European Patent Application EP 4 234 567 A1, published August 30, 2023. Title: Oligonucleotides for synthesizing 5'-capped RNA. Applicant: ST Pharm Co., Ltd. The sequence listing filed with the application follows.

SEQUENCE LISTING (3 sequences)

SEQ ID NO: 1 - DNA, 42 bp, Artificial Sequence
  forward primer
ttttttttctagaggtacctaatacgactcactataagcttg

SEQ ID NO: 2 - DNA, 35 bp, Artificial Sequence
  reverse primer
ttttttttggatccgagctcttacttgtacagctc

SEQ ID NO: 3 - DNA, 1083 bp, Artificial Sequence
  GFP DNA template
taatacgactcactataagcttgttctttttgcagaagctcagaataaacgctcaactttgggccaccatggtgagcaagggcgaggagctgttcaccggggtggtgcccatcctggtcgagctggacggcgacgtaaacggccacaagttcagcgtgtccggcgagggcgagggcgatgccacctacggcaagctgaccctgaagttcatctgcaccaccggcaagctgcccgtgccctggcccaccctcgtgaccaccctgacctacggcgtgcagtgcttcagccgctaccccgaccacatgaagcagcacgacttcttcaagtccgccatgcccgaaggctacgtccaggagcgcaccatcttcttcaaggacgacggcaactacaagacccgcgccgaggtgaagttcgagggcgacaccctggtgaaccgcatcgagctgaagggcatcgacttcaaggaggacggcaacatcctggggcacaagctggagtacaactacaacagccacaacgtctatatcatggccgacaagcagaagaacggcatcaaggtgaacttcaagatccgccacaacatcgaggacggcagcgtgcagctcgccgaccactaccagcagaacacccccatcggcgacggccccgtgctgctgcccgacaaccactacctgagcacccagtccgccctgagcaaagaccccaacgagaagcgcgatcacatggtcctgctggagttcgtgaccgccgccgggatcactctcggcatggacgagctgtacaagtaagagctcggatccaagcttctgcaggcatgcaaccagcctcaagaacacccgaatggagtctctaagctacataataccaacttacactttacaaaatgttgtcccccaaaatgtagccattcgtatctgctcctaataaaaagaaagtttcttcacaaaaaaaaaaaaaaaaaaaaaaaaaaaaaaaaaaaaaaaaaaaaaaaaaaaaaaaaaaaaaaaaaaaaaaaaaaaaaaaaaaaaaaaaaaaaaaaaaaaaaaaaaaaaaaaaaaaaaaaaaaaaaaaaaaaaaaaaccc